European Patent Specification EP 3 963 332 B1, published October 9, 2024. Title: Biomarkers for Disease Progression in Squamous Cell Carcinoma. Applicant: AMLo Biosciences LTD. The sequence listing filed with the application follows.

SEQUENCE LISTING (71 sequences)

SEQ ID NO: 1 - protein, 5 aa, Artificial Sequence
  HCDR1 of the anti-Ambra-1 antibody AbD33473
SYWIH

SEQ ID NO: 2 - protein, 17 aa, Artificial Sequence
  HCDR2 of the anti-Ambra-1 antibody AbD33473
TIFPSRSYTTYSPSFQG

SEQ ID NO: 3 - protein, 13 aa, Artificial Sequence
  HCDR3 of the anti-Ambra-1 antibody AbD33473
DTPSTALKSPFDY

SEQ ID NO: 4 - protein, 13 aa, Artificial Sequence
  LCDR1 of the anti-Ambra-1 antibody AbD33473
SGSSSNIGYNYVY

SEQ ID NO: 5 - protein, 7 aa, Artificial Sequence
  LCDR2 of the anti-Ambra-1 antibody AbD33473
ENNKRPS

SEQ ID NO: 6 - protein, 11 aa, Artificial Sequence
  LCDR3 of the anti-Ambra-1 antibody AbD33473
SSWDSHSNSYV

SEQ ID NO: 7 - protein, 30 aa, Artificial Sequence
  HCFR1 of the anti-Ambra-1 antibody AbD33473
EVQLVQSGAEVKKPGESLKISCKGSGYSFS

SEQ ID NO: 8 - protein, 14 aa, Artificial Sequence
  HCFR2 of the anti-Ambra-1 antibody AbD33473
WVRQMPGKGLEWMG

SEQ ID NO: 9 - protein, 32 aa, Artificial Sequence
  HCFR3 of the anti-Ambra-1 antibody AbD33473
QVTISADKSISTAYLQWSSLKASDTAMYYCAR

SEQ ID NO: 10 - protein, 11 aa, Artificial Sequence
  HCFR4 of the anti-Ambra-1 antibody AbD33473
WGQGTLVTVSS

SEQ ID NO: 11 - protein, 22 aa, Artificial Sequence
  LCFR1 of the anti-Ambra-1 antibody AbD33473
DIVLTQPPSVSGAPGQRVTISC

SEQ ID NO: 12 - protein, 15 aa, Artificial Sequence
  LCFR2 of the anti-Ambra-1 antibody AbD33473
WYQQLPGTAPKLLIY

SEQ ID NO: 13 - protein, 32 aa, Artificial Sequence
  LCFR3 of the anti-Ambra-1 antibody AbD33473
GVPDRFSGSKSGTSASLAITGLQAEDEADYYC

SEQ ID NO: 14 - protein, 12 aa, Artificial Sequence
  LCFR4 of the anti-Ambra-1 antibody AbD33473
FGGGTKLTVLGQ

SEQ ID NO: 15 - protein, 122 aa, Artificial Sequence
  VH domain of the anti-Ambra-1 antibody AbD33473
EVQLVQSGAEVKKPGESLKISCKGSGYSFSSYWIHWVRQMPGKGLEWMGTIFPSRSYTTYSPSFQGQVTISADKSISTAYLQWSSLKASDTAMYYCARDTPSTALKSPFDYWGQGTLVTVSS

SEQ ID NO: 16 - protein, 112 aa, Artificial Sequence
  VL domain of the anti-Ambra-1 antibody AbD33473
DIVLTQPPSVSGAPGQRVTISCSGSSSNIGYNYVYWYQQLPGTAPKLLIYENNKRPSGVPDRFSGSKSGTSASLAITGLQAEDEADYYCSSWDSHSNSYVFGGGTKLTVLGQ

SEQ ID NO: 17 - protein, 224 aa, Artificial Sequence
  Fd chain (VH domain and constant domain) of the Fab region of the anti-Ambra-1 antibody AbD33473
EVQLVQSGAEVKKPGESLKISCKGSGYSFSSYWIHWVRQMPGKGLEWMGTIFPSRSYTTYSPSFQGQVTISADKSISTAYLQWSSLKASDTAMYYCARDTPSTALKSPFDYWGQGTLVTVSSASTKGPSVFPLAPSSKSTSGGTAALGCLVKDYFPEPVTVSWNSGALTSGVHTFPAVLQSSGLYSLSSVVTVPSSSLGTQTYICNVNHKPSNTKVDKKVEPKS

SEQ ID NO: 18 - protein, 215 aa, Artificial Sequence
  light chain (VL domain and constant domain) of the Fab region of the anti-Ambra-1 antibody AbD33473
DIVLTQPPSVSGAPGQRVTISCSGSSSNIGYNYVYWYQQLPGTAPKLLIYENNKRPSGVPDRFSGSKSGTSASLAITGLQAEDEADYYCSSWDSHSNSYVFGGGTKLTVLGQPKAAPSVTLFPPSSEELQANKATLVCLISDFYPGAVTVAWKADSSPVKAGVETTTPSKQSNNKYAASSYLSLTPEQWKSHRSYSCQVTHEGSTVEKTVAPTEA

SEQ ID NO: 19 - DNA, 2085 bp, Artificial Sequence
  Fd chain of the Fab region and tags (alkaline phosphatase dimerization domain sequence (AP), FLAG tag (DYKDDDDK) and His6 tag of the anti-Ambra-1 antibody AbD33473
gaagtgcaattggtgcagagcggtgcggaagtgaaaaaaccgggcgaaagcctgaaaattagctgcaaaggctccggatatagcttctcttcttactggatccattgggtgcgccagatgccgggcaaaggtctcgagtggatgggcactatcttcccgtctcgtagctacaccacttatagcccgagctttcagggccaggtgaccattagcgcggataaaagcatcagcaccgcgtatctgcaatggagcagcctgaaagcgagcgataccgcgatgtattattgcgcgcgtgacactccgtctactgctctgaaatctccgttcgattactggggccaaggcaccctggtgactgttagctcagcgtcgaccaaaggcccgagcgtgtttccgctggccccgagcagcaaaagcaccagcggcggcaccgccgcactgggctgcctggtgaaagattatttcccggaaccagtgaccgtgagctggaacagcggtgccctgaccagcggcgtgcatacctttccggcggtgctgcaaagcagcggcctgtatagcctgagcagcgttgtgaccgtgccgagcagcagcctgggcacccagacctatatttgcaacgtcaaccataaaccgagcaacaccaaagtcgataaaaaagtcgaaccgaaaagcgaattcaaggctgaaatgcctgttctggaaaaccgggctgctcagggcgatattactacacccggcggtgctcgccgtttaacgggtgatcagactgccgctctgcgtgattctcttagcgataaacctgcaaaaaatattattttgctgattggcgatgggatgggggactcggaaattactgccgcacgtaattatgccgaaggtgcgggcggcttttttaaaggtatagatgccttaccgcttaccgggcaatacactcactatgcgctgaatagaaaaaccggcaaaccggactacgtcaccagctcggctgcatcagcaaccgcctggtcaaccggtgtcaaaacctataacggcgcgctgggcgtcgatattcacgaaaaagatcacccaacgattctggaaatggcaaaagccgcaggtctggcgaccggtaacgtttctaccgcagagttgcaggatgccacgcccgctgcgctggtggcacatgtgacctcgcgcaaatgctacggtccgagcgcgaccagtgaaaaatgtccgggtaacgctctggaaaaaggcggaaaaggatcgattaccgaacagctgcttaacgctcgtgccgacgttacgcttggcggcggcgcaaaaacctttgctgaaacggcaaccgctggtgaatggcagggaaaaacgctgcgtgaacaggcacaggcgcgtggttatcagttggtgagcgatgctgcctcactgaactcggtgacggaagcgaatcagcaaaaacccctgcttggcctgtttgctgacggcaatatgccagtgcgctggctaggaccgaaagcaacgtaccatggcaatatcgataagcccgcagtcacctgtacgccaaatccgcaacgtaatgacagtgtaccaaccctggcgcagatgaccgacaaagccattgaattgttgagtaaaaatgagaaaggctttttcctgcaagttgaaggtgcgtcaatcgataaacaggatcatgctgcgaatccttgtgggcaaattggcgagacggtcgatctcgatgaagccgtacaacgggcgctggagttcgctaaaaaggagggtaacacgctggtcatagtcaccgctgatcacgcccacgccagccagattgttgcgccggataccaaagctccgggcctcacccaggcgctaaataccaaagatggcgcagtgatggtgatgagttacgggaactccgaagaggattcacaagaacataccggcagtcagttgcgtattgcggcgtatggcccgcatgccgccaatgttgttggactgaccgaccagaccgatctcttctacaccatgaaagccgctctggggctgaaaggcgcgccggactataaagatgacgatgacaaaggcgcgccgcaccatcatcaccatcac

SEQ ID NO: 20 - DNA, 645 bp, Artificial Sequence
  Light chain of the Fab region of the anti-Ambra-1 antibody AbD33473
gatatcgtgctgacccagccgccgagcgtgagcggtgcaccgggccagcgcgtgaccattagctgtagcggcagcagcagcaacattggttacaactacgtgtactggtaccagcagctgccgggcacggcgccgaaactgctgatctacgaaaacaacaaacgcccgagcggcgtgccggatcgctttagcggatccaaaagcggcaccagcgccagcctggcgattaccggcctgcaagcagaagacgaagcggattattactgctcttcttgggactctcattctaactcttacgtgtttggcggcggcacgaagttaaccgttcttggccagccgaaagccgccccaagcgtgaccctgtttccgccgagcagcgaagaactgcaagccaacaaagccaccctggtttgcctgatcagcgatttttatccgggtgccgtgaccgtggcctggaaagccgatagcagcccggtgaaagccggcgtggaaaccaccaccccgagcaaacagagcaacaacaaatatgccgccagcagctatctgagcctgaccccggaacagtggaaaagccatcgcagctatagttgtcaagtgacccatgaaggcagcaccgtggaaaaaaccgtggccccgaccgaggcc

SEQ ID NO: 21 - protein, 1298 aa, Homo sapiens
MKVVPEKNAVRILWGRERGARAMGAQRLLQELVEDKTRWMKWEGKRVELPDSPRSTFLLAFSPDRTLLASTHVNHNIYITEVKTGKCVHSLIGHRRTPWCVTFHPTISGLIASGCLDGEVRIWDLHGGSESWFTDSNNAIASLAFHPTAQLLLIATANEIHFWDWSRREPFAVVKTASEMERVRLVRFDPLGHYLLTAIVNPSNQQGDDEPEIPIDGTELSHYRQRALLQSQPVRRTPLLHNFLHMLSSRSSGIQVGEQSTVQDSATPSPPPPPPQPSTERPRTSAYIRLRQRVSYPTAECCQHLGILCLCSRCSGTRVPSLLPHQDSVPPASARATTPSFSFVQTEPFHPPEQASSTQQDQGLLNRPSAFSTVQSSTAGNTLRNLSLGPTRRSLGGPLSSHPSRYHREIAPGLTGSEWTRTVLSLNSRSEAESMPPPRTSASSVSLLSVLRQQEGGSQASVYTSATEGRGFPASGLATESDGGNGSSQNNSGSIRHELQCDLRRFFLEYDRLQELDQSLSGEAPQTQQAQEMLNNNIESERPGPSHQPTPHSSENNSNLSRGHLNRCRACHNLLTFNNDTLRWERTTPNYSSGEASSSWQVPSSFESVPSSGSQLPPLERTEGQTPSSSRLELSSSASPQEERTVGVAFNQETGHWERIYTQSSRSGTVSQEALHQDMPEESSEEDSLRRRLLESSLISLSRYDGAGSREHPIYPDPARLSPAAYYAQRMIQYLSRRDSIRQRSMRYQQNRLRSSTSSSSSDNQGPSVEGTDLEFEDFEDNGDRSRHRAPRNARMSAPSLGRFVPRRFLLPEYLPYAGIFHERGQPGLATHSSVNRVLAGAVIGDGQSAVASNIANTTYRLQWWDFTKFDLPEISNASVNVLVQNCKIYNDASCDISADGQLLAAFIPSSQRGFPDEGILAVYSLAPHNLGEMLYTKRFGPNAISVSLSPMGRYVMVGLASRRILLHPSTEHMVAQVFRLQQAHGGETSMRRVFNVLYPMPADQRRHVSINSARWLPEPGLGLAYGTNKGDLVICRPEALNSGVEYYWDQLNETVFTVHSNSRSSERPGTSRATWRTDRDMGLMNAIGLQPRNPATSVTSQGTQTLALQLQNAETQTEREVPEPGTAASGPGEGEGSEYGASGEDALSRIQRLMAEGGMTAVVQREQSTTMASMGGFGNNIIVSHRIHRSSQTGTEPGAAHTSSPQPSTSRGLLPEAGQLAERGLSPRTASWDQPGTPGREPTQPTLPSSSPVPIPVSLPSAEGPTLHCELTNNNHLLDGGSSRGDAAGPRGEPRNR

SEQ ID NO: 22 - protein, 19 aa, Artificial Sequence
  peptide to which anti-Ambra-1 antibodies were raised
CGGSSRGDAAGPRGEPRNR

SEQ ID NO: 23 - protein, 5 aa, Artificial Sequence
  HCDR1 of anti-p62 antibody AbD34907
TYYLH

SEQ ID NO: 24 - protein, 17 aa, Artificial Sequence
  HCDR2 of the anti-p62 antibody AbD34907
LINPNNGGTNYAQKFQG

SEQ ID NO: 25 - protein, 14 aa, Artificial Sequence
  HCDR3 of the anti-p62 antibody AbD34907
GPGRLRPFGLYFDV

SEQ ID NO: 26 - protein, 11 aa, Artificial Sequence
  LCDR1 of the anti-p62 antibody AbD34907
RASQGIYTFLN

SEQ ID NO: 27 - protein, 7 aa, Artificial Sequence
  LCDR2 of the anti-p62 antibody AbD34907
AASTLQS

SEQ ID NO: 28 - protein, 9 aa, Artificial Sequence
  LCDR3 of the anti-p62 antibody AbD34907
FQYSSWPRT

SEQ ID NO: 29 - protein, 30 aa, Artificial Sequence
  HCFR1 of the anti-p62 antibody AbD34907
QVQLVQSGAEVKKPGASVKVSCKASGYTFN

SEQ ID NO: 30 - protein, 14 aa, Artificial Sequence
  HCFR2 of the anti-p62 antibody AbD34907
WVRQAPGQGLEWMG

SEQ ID NO: 31 - protein, 32 aa, Artificial Sequence
  HCFR3 of the anti-p62 antibody AbD34907
RVTMTRDTSISTAYMELSRLRSEDTAVYYCAR

SEQ ID NO: 32 - protein, 11 aa, Artificial Sequence
  HCFR4 of the anti-p62 antibody AbD34907
WGQGTLVTVSS

SEQ ID NO: 33 - protein, 23 aa, Artificial Sequence
  LCFR1 of the anti-p62 antibody AbD34907
DIQMTQSPSSLSASVGDRVTITC

SEQ ID NO: 34 - protein, 15 aa, Artificial Sequence
  LCFR2 of the anti-p62 antibody AbD34907
WYQQKPGKAPKLLIY

SEQ ID NO: 35 - protein, 32 aa, Artificial Sequence
  LCFR3 of the anti-p62 antibody AbD34907
GVPSRFSGSGSGTDFTLTISSLQPEDFATYYC

SEQ ID NO: 36 - protein, 10 aa, Artificial Sequence
  LCFR4 of the anti-p62 antibody AbD34907
FGQGTKVEIK

SEQ ID NO: 37 - protein, 123 aa, Artificial Sequence
  VH domain of the anti-p62 antibody AbD34907
QVQLVQSGAEVKKPGASVKVSCKASGYTFNTYYLHWVRQAPGQGLEWMGLINPNNGGTNYAQKFQGRVTMTRDTSISTAYMELSRLRSEDTAVYYCARGPGRLRPFGLYFDVWGQGTLVTVSS

SEQ ID NO: 38 - protein, 107 aa, Artificial Sequence
  VL domain of the anti-p62 antibody AbD34907
DIQMTQSPSSLSASVGDRVTITCRASQGIYTFLNWYQQKPGKAPKLLIYAASTLQSGVPSRFSGSGSGTDFTLTISSLQPEDFATYYCFQYSSWPRTFGQGTKVEIK

SEQ ID NO: 39 - protein, 225 aa, Artificial Sequence
  Fd chain (VH domain and constant domain) of the Fab region of the anti-p62 antibody AbD34907
QVQLVQSGAEVKKPGASVKVSCKASGYTFNTYYLHWVRQAPGQGLEWMGLINPNNGGTNYAQKFQGRVTMTRDTSISTAYMELSRLRSEDTAVYYCARGPGRLRPFGLYFDVWGQGTLVTVSSASTKGPSVFPLAPSSKSTSGGTAALGCLVKDYFPEPVTVSWNSGALTSGVHTFPAVLQSSGLYSLSSVVTVPSSSLGTQTYICNVNHKPSNTKVDKKVEPKS

SEQ ID NO: 40 - protein, 214 aa, Artificial Sequence
  Light chain (VL domain and constant domain) of the Fab region of the anti-p62 antibody AbD34907
DIQMTQSPSSLSASVGDRVTITCRASQGIYTFLNWYQQKPGKAPKLLIYAASTLQSGVPSRFSGSGSGTDFTLTISSLQPEDFATYYCFQYSSWPRTFGQGTKVEIKRTVAAPSVFIFPPSDEQLKSGTASVVCLLNNFYPREAKVQWKVDNALQSGNSQESVTEQDSKDSTYSLSSTLTLSKADYEKHKVYACEVTHQGLSSPVTKSFNRGEA

SEQ ID NO: 41 - protein, 5 aa, Artificial Sequence
  HCDR1 of anti-p62 antibody AbD34908
NYWIG

SEQ ID NO: 42 - protein, 17 aa, Artificial Sequence
  HCDR2 of the anti-p62 antibody AbD34908
IIDPSGSFTRYSPSFQG

SEQ ID NO: 43 - protein, 17 aa, Artificial Sequence
  HCDR3 of the anti-p62 antibody AbD34908
KYVPPVYSYWSYGTLDV

SEQ ID NO: 44 - protein, 12 aa, Artificial Sequence
  LCDR1 of the anti-p62 antibody AbD34908
RASQSVSASRLA

SEQ ID NO: 45 - protein, 7 aa, Artificial Sequence
  LCDR2 of the anti-p62 antibody AbD34908
GSSTRAT

SEQ ID NO: 46 - protein, 8 aa, Artificial Sequence
  LCDR3 of the anti-p62 antibody AbD34908
QQYLHLYT

SEQ ID NO: 47 - protein, 30 aa, Artificial Sequence
  HCFR1 of the anti-p62 antibody AbD34908
EVQLVQSGAEVKKPGESLKISCKGSGYSFT

SEQ ID NO: 48 - protein, 14 aa, Artificial Sequence
  HCFR2 of the anti-p62 antibody AbD34908
WVRQMPGKGLEWMG

SEQ ID NO: 49 - protein, 32 aa, Artificial Sequence; identical to SEQ ID NO: 9
  HCFR3 of the anti-p62 antibody AbD34908

SEQ ID NO: 50 - protein, 11 aa, Artificial Sequence
  HCFR4 of the anti-p62 antibody AbD34908
WGQGTLVTVSS

SEQ ID NO: 51 - protein, 23 aa, Artificial Sequence
  LCFR1 of the anti-p62 antibody AbD34908
DIVLTQSPATLSLSPGERATLSC

SEQ ID NO: 52 - protein, 15 aa, Artificial Sequence
  LCFR2 of the anti-p62 antibody AbD34908
WYQQKPGQAPRLLIY

SEQ ID NO: 53 - protein, 32 aa, Artificial Sequence
  LCFR3 of the anti-p62 antibody AbD34908
GIPARFSGSGSGTDFTLTISSLEPEDFAVYYC

SEQ ID NO: 54 - protein, 10 aa, Artificial Sequence
  LCFR4 of the anti-p62 antibody AbD34908
FGQGTKVEIK

SEQ ID NO: 55 - protein, 126 aa, Artificial Sequence
  VH domain of the anti-p62 antibody AbD34908
EVQLVQSGAEVKKPGESLKISCKGSGYSFTNYWIGWVRQMPGKGLEWMGIIDPSGSFTRYSPSFQGQVTISADKSISTAYLQWSSLKASDTAMYYCARKYVPPVYSYWSYGTLDVWGQGTLVTVSS

SEQ ID NO: 56 - protein, 107 aa, Artificial Sequence
  VL domain of the anti-p62 antibody AbD34908
DIVLTQSPATLSLSPGERATLSCRASQSVSASRLAWYQQKPGQAPRLLIYGSSTRATGIPARFSGSGSGTDFTLTISSLEPEDFAVYYCQQYLHLYTFGQGTKVEIK

SEQ ID NO: 57 - protein, 228 aa, Artificial Sequence
  Fd chain (VH domain and constant domain) of the Fab region of the anti-p62 antibody AbD34908
EVQLVQSGAEVKKPGESLKISCKGSGYSFTNYWIGWVRQMPGKGLEWMGIIDPSGSFTRYSPSFQGQVTISADKSISTAYLQWSSLKASDTAMYYCARKYVPPVYSYWSYGTLDVWGQGTLVTVSSASTKGPSVFPLAPSSKSTSGGTAALGCLVKDYFPEPVTVSWNSGALTSGVHTFPAVLQSSGLYSLSSVVTVPSSSLGTQTYICNVNHKPSNTKVDKKVEPKS

SEQ ID NO: 58 - protein, 214 aa, Artificial Sequence
  light chain (VL domain and constant domain) of the Fab region of the anti-p62 antibody AbD34908
DIVLTQSPATLSLSPGERATLSCRASQSVSASRLAWYQQKPGQAPRLLIYGSSTRATGIPARFSGSGSGTDFTLTISSLEPEDFAVYYCQQYLHLYTFGQGTKVEIKRTVAAPSVFIFPPSDEQLKSGTASVVCLLNNFYPREAKVQWKVDNALQSGNSQESVTEQDSKDSTYSLSSTLTLSKADYEKHKVYACEVTHQGLSSPVTKSFNRGEA

SEQ ID NO: 59 - protein, 910 aa, Artificial Sequence
  Full amino acid sequence of the anti-p62 antibody AbD34907 including alkaline phosphatase dimerization domain sequence (AP), FLAG and His6 tag
DIQMTQSPSSLSASVGDRVTITCRASQGIYTFLNWYQQKPGKAPKLLIYAASTLQSGVPSRFSGSGSGTDFTLTISSLQPEDFATYYCFQYSSWPRTFGQGTKVEIKRTVAAPSVFIFPPSDEQLKSGTASVVCLLNNFYPREAKVQWKVDNALQSGNSQESVTEQDSKDSTYSLSSTLTLSKADYEKHKVYACEVTHQGLSSPVTKSFNRGEAQVQLVQSGAEVKKPGASVKVSCKASGYTFNTYYLHWVRQAPGQGLEWMGLINPNNGGTNYAQKFQGRVTMTRDTSISTAYMELSRLRSEDTAVYYCARGPGRLRPFGLYFDVWGQGTLVTVSSASTKGPSVFPLAPSSKSTSGGTAALGCLVKDYFPEPVTVSWNSGALTSGVHTFPAVLQSSGLYSLSSVVTVPSSSLGTQTYICNVNHKPSNTKVDKKVEPKSEFKAEMPVLENRAAQGDITTPGGARRLTGDQTAALRDSLSDKPAKNIILLIGDGMGDSEITAARNYAEGAGGFFKGIDALPLTGQYTHYALNRKTGKPDYVTSSAASATAWSTGVKTYNGALGVDIHEKDHPTILEMAKAAGLATGNVSTAELQDATPAALVAHVTSRKCYGPSATSEKCPGNALEKGGKGSITEQLLNARADVTLGGGAKTFAETATAGEWQGKTLREQAQARGYQLVSDAASLNSVTEANQQKPLLGLFADGNMPVRWLGPKATYHGNIDKPAVTCTPNPQRNDSVPTLAQMTDKAIELLSKNEKGFFLQVEGASIDKQDHAANPCGQIGETVDLDEAVQRALEFAKKEGNTLVIVTADHAHASQIVAPDTKAPGLTQALNTKDGAVMVMSYGNSEEDSQEHTGSQLRIAAYGPHAANVVGLTDQTDLFYTMKAALGLKGAPDYKDDDDKGAPHHHHHH

SEQ ID NO: 60 - protein, 913 aa, Artificial Sequence
  Full amino acid sequence of the anti-p62 antibody AbD34908 including alkaline phosphatase dimerization domain sequence (AP), FLAG and His6 tag
DIVLTQSPATLSLSPGERATLSCRASQSVSASRLAWYQQKPGQAPRLLIYGSSTRATGIPARFSGSGSGTDFTLTISSLEPEDFAVYYCQQYLHLYTFGQGTKVEIKRTVAAPSVFIFPPSDEQLKSGTASVVCLLNNFYPREAKVQWKVDNALQSGNSQESVTEQDSKDSTYSLSSTLTLSKADYEKHKVYACEVTHQGLSSPVTKSFNRGEAEVQLVQSGAEVKKPGESLKISCKGSGYSFTNYWIGWVRQMPGKGLEWMGIIDPSGSFTRYSPSFQGQVTISADKSISTAYLQWSSLKASDTAMYYCARKYVPPVYSYWSYGTLDVWGQGTLVTVSSASTKGPSVFPLAPSSKSTSGGTAALGCLVKDYFPEPVTVSWNSGALTSGVHTFPAVLQSSGLYSLSSVVTVPSSSLGTQTYICNVNHKPSNTKVDKKVEPKSEFKAEMPVLENRAAQGDITTPGGARRLTGDQTAALRDSLSDKPAKNIILLIGDGMGDSEITAARNYAEGAGGFFKGIDALPLTGQYTHYALNRKTGKPDYVTSSAASATAWSTGVKTYNGALGVDIHEKDHPTILEMAKAAGLATGNVSTAELQDATPAALVAHVTSRKCYGPSATSEKCPGNALEKGGKGSITEQLLNARADVTLGGGAKTFAETATAGEWQGKTLREQAQARGYQLVSDAASLNSVTEANQQKPLLGLFADGNMPVRWLGPKATYHGNIDKPAVTCTPNPQRNDSVPTLAQMTDKAIELLSKNEKGFFLQVEGASIDKQDHAANPCGQIGETVDLDEAVQRALEFAKKEGNTLVIVTADHAHASQIVAPDTKAPGLTQALNTKDGAVMVMSYGNSEEDSQEHTGSQLRIAAYGPHAANVVGLTDQTDLFYTMKAALGLKGAPDYKDDDDKGAPHHHHHH

SEQ ID NO: 61 - protein, 440 aa, Homo sapiens
MASLTVKAYLLGKEDAAREIRRFSFCCSPEPEAEAEAAAGPGPCERLLSRVAALFPALRPGGFQAHYRDEDGDLVAFSSDEELTMAMSYVKDDIFRIYIKEKKECRRDHRPPCAQEAPRNMVHPNVICDGCNGPVVGTRYKCSVCPDYDLCSVCEGKGLHRGHTKLAFPSPFGHLSEGFSHSRWLRKVKHGHFGWPGWEMGPPGNWSPRPPRAGEARPGPTAESASGPSEDPSVNFLKNVGESVAAALSPLGIEVDIDVEHGGKRSRLTPVSPESSSTEEKSSSQPSSCCSDPSKPGGNVEGATQSLAEQMRKIALESEGRPEEQMESDNCSGGDDDWTHLSSKEVDPSTGELQSLQMPESEGPSSLDPSQEGPTGLKEAALYPHLPPEADPRLIESLSQMLSMGFSDEGGWLTRLLQTKNYDIGAALDTIQYSKHPPPL

SEQ ID NO: 62 - protein, 364 aa, Artificial Sequence
  p62 protein fragment used to generate anti-p62 antibodies
MAMSYVKDDIFRIYIKEKKECRRDHRPPCAQEAPRNMVHPNVICDGCNGPVVGTRYKCSVCPDYDLCSVCEGKGLHRGHTKLAFPSPFGHLSEGFSHSRWLRKVKHGHFGWPGWEMGPPGNWSPRPPRAGEARPGPTAESASGPSEDPSVNFLKNVGESVAAALSPLGIEVDIDVEHGGKRSRLTPVSPESSSTEEKSSSQPSSCCSDPSKPGGNVEGATQSLAEQMRKIALESEGRPEEQMESDNCSGGDDDWTHLSSKEVDPSTGELQSLQMPESEGPSSLDPSQEGPTGLKEAALYPHLPPEADPRLIESLSQMLSMGFSDEGGWLTRLLQTKNYDIGAALDTIQYSKHPPPLLEHHHHHH

SEQ ID NO: 63 - protein, 41 aa, Artificial Sequence
  Ambra-1 C-terminal sequence used for replacement analysis in epitope mapping
VSLPSAEGPTLHCELTNNNHLLDGGSSRGDAAGPRGEPRNR

SEQ ID NO: 64 - protein, 19 aa, Artificial Sequence
  REPNET epitope of the Anti-Ambra-1 antibodies
DGGSSRGDAAGPRGEPRNR

SEQ ID NO: 65 - protein, 9 aa, Artificial Sequence
  LIN epitope of the Anti-Ambra-1 antibodies
HLLDGGSSR

SEQ ID NO: 66 - protein, 10 aa, Artificial Sequence
  LOOP epitope of the Anti-Ambra-1 antibodies
NHLLDGGSSR

SEQ ID NO: 67 - protein, 4 aa, Artificial Sequence
  core epitope of the Anti-Ambra-1 antibodies
EPRN

SEQ ID NO: 68 - skipped

SEQ ID NO: 69 - protein, 8 aa, Artificial Sequence
  EPITOPE TAG
DYKDDDDK

SEQ ID NO: 70 - protein, 14 aa, Artificial Sequence
  EPITOPE TAG
GKPIPNPLLGLDST

SEQ ID NO: 71 - protein, 8 aa, Artificial Sequence
  EPITOPE TAG
WSHPQFEK